European Patent Application EP 4 144 898 A1, published March 8, 2023. Title: Verfahren zur Selektion oder Screenen von Antikörpern aus einer Antikörperbibliothek. Applicant: new/era/mabs GmbH. The sequence listing filed with the application follows.

SEQUENCE LISTING (20 sequences)

SEQ ID NO: 1 - protein, 15 aa, AviTag Artificial
GLNDIFEAQKIEWHE

SEQ ID NO: 2 - protein, 13 aa, AviTag Artificial
LNDIFEAQKIEWH

SEQ ID NO: 3 - protein, 13 aa, Artificial
  Biotinylation
  MISC_FEATURE (2)..(2): Xaa can be N, C or any amino acid or be deleted
  MISC_FEATURE (3)..(3): Xaa can be any amino acid except L, V, I, W, F, Y
  MISC_FEATURE (5)..(5): Xaa can be F or L
  MISC_FEATURE (6)..(6): Xaa can be E or D
  MISC_FEATURE (7)..(7): Xaa can be A, G, S, T
  MISC_FEATURE (8)..(8): Xaa can be Q or M
  MISC_FEATURE (10)..(10): Xaa can be I, M, V
  MISC_FEATURE (11)..(11): Xaa can be E, L, V, Y, I
  MISC_FEATURE (12)..(12): Xaa can be W,Y,V,F,L, I
  MISC_FEATURE (13)..(13): Xaa can be R,H or any amino acid except D, E
LXXIXXXXKXXXX

SEQ ID NO: 4 - protein, 4 aa, No
KDEL

SEQ ID NO: 5 - DNA, 27 bp, HA-Tag artificial
tatccatatgatgttccagattatgct

SEQ ID NO: 6 - protein, 9 aa, HA-Tag artificial
YPYDVPDYA

SEQ ID NO: 7 - DNA, 45 bp, AviTag artificial
ggcctgaacgacatcttcgaggcccagaagatcgagtggcacgag

SEQ ID NO: 8 - DNA, 72 bp, Human (EGFR Signal)
atgcgaccctccgggacggccggggcagcgctcctggcgctgctggctgcgctctgcccggcgagtcgggct

SEQ ID NO: 9 - protein, 24 aa, Human (EGFR-Signal)
MRPSGTAGAALLALLAALCPASRA

SEQ ID NO: 10 - DNA, 1956 bp, Human (EGFR)
ctggaggaaaagaaagtttgccaaggcacgagtaacaagctcacgcagttgggcacttttgaagatcattttctcagcctccagaggatgttcaataactgtgaggtggtccttgggaatttggaaattacctatgtgcagaggaattatgatctttccttcttaaagaccatccaggaggtggctggttatgccctcattgccctcaacacagtggagcgaattcctttggaaaacctgcagatcatcagaggaaatatgtactacgaaaattcctatgccttagcagtcttatctaactatgatgcaaataaaaccggactgaaggagctgcccatgagaaatttacaggaaatcctgcatggcgccgtgcggttcagcaacaaccctgccctgtgcaacgtggagagcatccagtggcgggacatagtcagcagtgactttctcagcaacatgtcgatggacttccagaaccacctgggcagctgccaaaagtgtgatccaagctgtcccaatgggagctgctggggtgcaggagaggagaactgccagagactgaccaaaatcatctgtgcccagcagtgctccgggcgctgccgtggcaagtcccccagtgactgctgccacaaccagtgtgctgcaggctgcacaggcccccgggagagcgactgcctggtctgccgcaaattccgagacgaagccacgtgcaaggacacctgccccccactcatgctctacaaccccaccacgtaccagatggatgtgaaccccgagggcaaatacagctttggtgccacctgcgtgaagaagtgtccccgtaattatgtggtgacagatcacggctcgtgcgtccgagcctgtggggccgacagctatgagatggaggaagacggcgtccgcaagtgtaagaagtgcgaagggccttgccgcaaagtgtgtaacggaataggtattggtgaatttaaagactcactctccataaatgctacgaatattaaacacttcaaaaactgcacctccatcagtggcgatctccacatcctgccggtggcatttaggggtgactccttcacacatactcctcctctggatccacaggaactggatattctgaaaaccgtaaaggaaatcacagggtttttgctgattcaggcttggcctgaaaacaggacggacctccatgcctttgagaacctagaaatcatacgcggcaggaccaagcaacatggtcagttttctcttgcagtcgtcagcctgaacataacatccttgggattacgctccctcaaggagataagtgatggagatgtgataatttcaggaaacaaaaatttgtgctatgcaaatacaataaactggaaaaaactgtttgggacctccggtcagaaaaccaaaattataagcaacagaggtgaaaacagctgcaaggccacaggccaggtctgccatgccttgtgctcccccgagggctgctggggcccggagcccagggactgcgtctcttgccggaatgtcagccgaggcagggaatgcgtggacaagtgcaaccttctggagggtgagccaagggagtttgtggagaactctgagtgcatacagtgccacccagagtgcctgcctcaggccatgaacatcacctgcacaggacggggaccagacaactgtatccagtgtgcccactacattgacggcccccactgcgtcaagacctgcccggcaggagtcatgggagaaaacaacaccctggtctggaagtacgcagacgccggccatgtgtgccacctgtgccatccaaactgcacctacggatgcactgggccaggtcttgaaggctgtccaacgaatgggcctaagatcccgtccatcgccactgggatggtgggggccctcctcttgctgctggtggtggccctggggatcggcctcttcatgcgaaggcgccacatcgttcggtaa

SEQ ID NO: 11 - protein, 651 aa, Human (EGFR)
LEEKKVCQGTSNKLTQLGTFEDHFLSLQRMFNNCEVVLGNLEITYVQRNYDLSFLKTIQEVAGYALIALNTVERIPLENLQIIRGNMYYENSYALAVLSNYDANKTGLKELPMRNLQEILHGAVRFSNNPALCNVESIQWRDIVSSDFLSNMSMDFQNHLGSCQKCDPSCPNGSCWGAGEENCQRLTKIICAQQCSGRCRGKSPSDCCHNQCAAGCTGPRESDCLVCRKFRDEATCKDTCPPLMLYNPTTYQMDVNPEGKYSFGATCVKKCPRNYVVTDHGSCVRACGADSYEMEEDGVRKCKKCEGPCRKVCNGIGIGEFKDSLSINATNIKHFKNCTSISGDLHILPVAFRGDSFTHTPPLDPQELDILKTVKEITGFLLIQAWPENRTDLHAFENLEIIRGRTKQHGQFSLAVVSLNITSLGLRSLKEISDGDVIISGNKNLCYANTINWKKLFGTSGQKTKIISNRGENSCKATGQVCHALCSPEGCWGPEPRDCVSCRNVSRGRECVDKCNLLEGEPREFVENSECIQCHPECLPQAMNITCTGRGPDNCIQCAHYIDGPHCVKTCPAGVMGENNTLVWKYADAGHVCHLCHPNCTYGCTGPGLEGCPTNGPKIPSIATGMVGALLLLLVVALGIGLFMRRRHIVR

SEQ ID NO: 12 - DNA, 552 bp, IRES artificial
acgttactggccgaagccgcttggaataaggccggtgtgcgtttgtctatatgttattttccaccatattgccgtcttttggcaatgtgagggcccggaaacctggccctgtcttcttgacgagcattcctaggggtctttcccctctcgccaaaggaatgcaaggtctgttgaatgtcgtgaaggaagcagttcctctggaagcttcttgaagacaaacaacgtctgtagcgaccctttgcaggcagcggaaccccccacctggcgacaggtgcctctgcggccaaaagccacgtgtataagatacacctgcaaaggcggcacaaccccagtgccacgttgtgagttggatagttgtggaaagagtcaaatggctctcctcaagcgtattcaacaaggggctgaaggatgcccagaaggtaccccattgtatgggatctgatctggggcctcggtgcacatgctttacatgtgtttagtcgaggttaaaaaaacgtctaggccccccgaaccacggggacgtggttttcctttgaaaaacacgatgataat

SEQ ID NO: 13 - DNA, 1005 bp, Escherichia coli
atgaaggataacaccgtgccactgaaattgattgccctgttagcgaacggtgaatttcactctggcgagcagttgggtgaaacgctgggaatgagccgggcggctattaataaacacattcagacactgcgtgactggggcgttgatgtctttaccgttccgggtaaaggatacagcctgcctgagcctatccagttacttaatgctaaacagatattgggtcagctggatggcggtagtgtagccgtgctgcctgtgattgactccacgaatcagtaccttcttgatcgtatcggagagcttaaatcgggcgatgcttgcattgcagaataccagcaggctggccgtggtcgccggggtcggaaatggttttcgccttttggcgcaaacttatatttgtcgatgttctggcgtctggaacaaggcccggcggcggcgattggtttaagtctggttatcggtatcgtgatggcggaagtattacgcaagctgggtgcagataaagttcgtgttaaatggcctaatgacctctatctgcaggatcgcaagctggcaggcattctggtggagctgactggcaaaactggcgatgcggcgcaaatagtcattggagccgggatcaacatggcaatgcgccgtgttgaagagagtgtcgttaatcaggggtggatcacgctgcaggaagcggggatcaatctcgatcgtaatacgttggcggccatgctaatacgtgaattacgtgctgcgttggaactcttcgaacaagaaggattggcaccttatctgtcgcgctgggaaaagctggataattttattaatcgcccagtgaaacttatcattggtgataaagaaatatttggcatttcacgcggaatagacaaacagggggctttattacttgagcaggatggaataataaaaccctggatgggcggtgaaatatccctgcgtagtgcagaaaaagggtctacatctggatctgggggttcaaaggacgagctgtga

SEQ ID NO: 14 - protein, 9 aa, No
YPYDVPDYA

SEQ ID NO: 15 - DNA, 12502 bp, expressionsvector
ctaaattgtaagcgttaatattttgttaaaattcgcgttaaatttttgttaaatcagctcattttttaaccaataggccgaaatcggcaaaatcccttataaatcaaaagaatagaccgagatagggttgagtgttgttccagtttggaacaagagtccactattaaagaacgtggactccaacgtcaaagggcgaaaaaccgtctatcagggcgatggcccactacgtgaaccatcaccctaatcaagttttttggggtcgaggtgccgtaaagcactaaatcggaaccctaaagggagcccccgatttagagcttgacggggaaagccggcgaacgtggcgagaaaggaagggaagaaagcgaaaggagcgggcgctagggcgctggcaagtgtagcggtcacgctgcgcgtaaccaccacacccgccgcgcttaatgcgccgctacagggcgcgtcccattcgccattcaggctgcgcaactgttgggaagggcgatcggtgcgggcctcttcgctattacgccagctggcgaaagggggatgtgctgcaaggcgattaagttgggtaacgccagggttttcccagtcacgacgttgtaaaacgacggccagtgagcgcgcgtaatacgactcactatagggcgaattggggcgcgccattctagattaaccctagaaagatagtctgcgtaaaattgacgcatgcattcttgaaatattgctctctctttctaaatagcgcgaatccgtcgctgtgcatttaggacatctcagtcgccgcttggagctcccgtgaggcgtgcttgtcaatgcggtaagtgtcactgattttgaactataacgaccgcgtgagtcaaaatgacgcatgattatcttttacgtgacttttaagatttaactcatacgataattatattgttatttcatgttctacttacgtgataacttattatatatatattttcttgttatagatatcaactagaatgctagcagatctcgaccgagctttgcaaagatggataaagttttaaacagagaggaatctttgcagctaatggaccttctaggtcttgaaaggagtgggaattggctccggtgcccgtcagtgggcagagcgcacatcgcccacagtccccgagaagttggggggaggggtcggcaattgaaccggtgcctagagaaggtggcgcggggtaaactgggaaagtgatgtcgtgtactggctccgcctttttcccgagggtgggggagaaccgtatataagtgcagtagtcgccgtgaacgttctttttcgcaacgggtttgccgccagaacacaggtaagtgccgtgtgtggttcccgcgggcctggcctctttacgggttatggcccttgcgtgccttgaattacttccacctggctgcagtacgtgattcttgatcccgagcttcgggttggaagtgggtgggagagttcgaggccttgcgcttaaggagccccttcgcctcgtgcttgagttgaggcctggcctgggcgctggggccgccgcgtgcgaatctggtggcaccttcgcgcctgtctcgctgctttcgataagtctctagccatttaaaatttttgatgacctgctgcgacgctttttttctggcaagatagtcttgtaaatgcgggccaagatcgatctgcacactggtatttcggtttttggggccgcgggcggcgacggggcccgtgcgtcccagcgcacatgttcggcgaggcggggcctgcgagcgcggccaccgagaatcggacgggggtagtctcaagctggccggcctgctctggtgcctggcctcgcgccgccgtgtatcgccccgccctgggcggcaaggctggcccggtcggcaccagttgcgtgagcggaaagatggccgcttcccggccctgctgcagggagctcaaaatggaggacgcggcgctcgggagagcgggcgggtgagtcacccacacaaaggaaaagggcctttccgtcctcagccgtcgcttcatgtgactccacggagtaccgggcgccgtccaggcacctcgattagttctcgatcgagcttttggagtacgtcgtctttaggttggggggaggggttttatgcgatggagtttccccacactgagtgggtggagactgaagttaggccagcttggcacttgatgtaattctccttggaatttgccctttttgagtttggatcttggttcattctcaagcctcagacagtggttcaaagtttttttcttccatttcaggtgtcgtgaggaattagcttgaccaagcttcgaattctgcagtcgacggtaccgccaccatgcgaccctccgggacggccggggcagcgctcctggcgctgctggctgcgctctgcccggcgagtcgggctctggaggaaggctcgtctaagcttggctcgtctgggtatccatatgatgttccagattatgctggggcccagccggccagatctggcggcggcctgaacgacatcttcgaggcccagaagatcgagtggcacgagggcgcgccggctaccggaagcagcgggctggaggaaaagaaagtttgccaaggcacgagtaacaagctcacgcagttgggcacttttgaagatcattttctcagcctccagaggatgttcaataactgtgaggtggtccttgggaatttggaaattacctatgtgcagaggaattatgatctttccttcttaaagaccatccaggaggtggctggttatgccctcattgccctcaacacagtggagcgaattcctttggaaaacctgcagatcatcagaggaaatatgtactacgaaaattcctatgccttagcagtcttatctaactatgatgcaaataaaaccggactgaaggagctgcccatgagaaatttacaggaaatcctgcatggcgccgtgcggttcagcaacaaccctgccctgtgcaacgtggagagcatccagtggcgggacatagtcagcagtgactttctcagcaacatgtcgatggacttccagaaccacctgggcagctgccaaaagtgtgatccaagctgtcccaatgggagctgctggggtgcaggagaggagaactgccagagactgaccaaaatcatctgtgcccagcagtgctccgggcgctgccgtggcaagtcccccagtgactgctgccacaaccagtgtgctgcaggctgcacaggcccccgggagagcgactgcctggtctgccgcaaattccgagacgaagccacgtgcaaggacacctgccccccactcatgctctacaaccccaccacgtaccagatggatgtgaaccccgagggcaaatacagctttggtgccacctgcgtgaagaagtgtccccgtaattatgtggtgacagatcacggctcgtgcgtccgagcctgtggggccgacagctatgagatggaggaagacggcgtccgcaagtgtaagaagtgcgaagggccttgccgcaaagtgtgtaacggaataggtattggtgaatttaaagactcactctccataaatgctacgaatattaaacacttcaaaaactgcacctccatcagtggcgatctccacatcctgccggtggcatttaggggtgactccttcacacatactcctcctctggatccacaggaactggatattctgaaaaccgtaaaggaaatcacagggtttttgctgattcaggcttggcctgaaaacaggacggacctccatgcctttgagaacctagaaatcatacgcggcaggaccaagcaacatggtcagttttctcttgcagtcgtcagcctgaacataacatccttgggattacgctccctcaaggagataagtgatggagatgtgataatttcaggaaacaaaaatttgtgctatgcaaatacaataaactggaaaaaactgtttgggacctccggtcagaaaaccaaaattataagcaacagaggtgaaaacagctgcaaggccacaggccaggtctgccatgccttgtgctcccccgagggctgctggggcccggagcccagggactgcgtctcttgccggaatgtcagccgaggcagggaatgcgtggacaagtgcaaccttctggagggtgagccaagggagtttgtggagaactctgagtgcatacagtgccacccagagtgcctgcctcaggccatgaacatcacctgcacaggacggggaccagacaactgtatccagtgtgcccactacattgacggcccccactgcgtcaagacctgcccggcaggagtcatgggagaaaacaacaccctggtctggaagtacgcagacgccggccatgtgtgccacctgtgccatccaaactgcacctacggatgcactgggccaggtcttgaaggctgtccaacgaatgggcctaagatcccgtccatcgccactgggatggtgggggccctcctcttgctgctggtggtggccctggggatcggcctcttcatgcgaaggcgccacatcgttcggtaagcggccgctctagcccaattccgcccccccccccctaacgttactggccgaagccgcttggaataaggccggtgtgcgtttgtctatatgttattttccaccatattgccgtcttttggcaatgtgagggcccggaaacctggccctgtcttcttgacgagcattcctaggggtctttcccctctcgccaaaggaatgcaaggtctgttgaatgtcgtgaaggaagcagttcctctggaagcttcttgaagacaaacaacgtctgtagcgaccctttgcaggcagcggaaccccccacctggcgacaggtgcctctgcggccaaaagccacgtgtataagatacacctgcaaaggcggcacaaccccagtgccacgttgtgagttggatagttgtggaaagagtcaaatggctctcctcaagcgtattcaacaaggggctgaaggatgcccagaaggtaccccattgtatgggatctgatctggggcctcggtgcacatgctttacatgtgtttagtcgaggttaaaaaaacgtctaggccccccgaaccacggggacgtggttttcctttgaaaaacacgatgataatatgggccgaccctccgggacggccggggcagcgctcctggcgctgctggctgcgctctgcccggcgagtcgggctctggaggaaggctcgtctaagcttggctcgtctgggatgaaggataacaccgtgccactgaaattgattgccctgttagcgaacggtgaatttcactctggcgagcagttgggtgaaacgctgggaatgagccgggcggctattaataaacacattcagacactgcgtgactggggcgttgatgtctttaccgttccgggtaaaggatacagcctgcctgagcctatccagttacttaatgctaaacagatattgggtcagctggatggcggtagtgtagccgtgctgcctgtgattgactccacgaatcagtaccttcttgatcgtatcggagagcttaaatcgggcgatgcttgcattgcagaataccagcaggctggccgtggtcgccggggtcggaaatggttttcgccttttggcgcaaacttatatttgtcgatgttctggcgtctggaacaaggcccggcggcggcgattggtttaagtctggttatcggtatcgtgatggcggaagtattacgcaagctgggtgcagataaagttcgtgttaaatggcctaatgacctctatctgcaggatcgcaagctggcaggcattctggtggagctgactggcaaaactggcgatgcggcgcaaatagtcattggagccgggatcaacatggcaatgcgccgtgttgaagagagtgtcgttaatcaggggtggatcacgctgcaggaagcggggatcaatctcgatcgtaatacgttggcggccatgctaatacgtgaattacgtgctgcgttggaactcttcgaacaagaaggattggcaccttatctgtcgcgctgggaaaagctggataattttattaatcgcccagtgaaacttatcattggtgataaagaaatatttggcatttcacgcggaatagacaaacagggggctttattacttgagcaggatggaataataaaaccctggatgggcggtgaaatatccctgcgtagtgcagaaaaagggtctacatctggatctgggggttcaaaggacgagctgtgactcgagtctagagggcccgtttaaacccgctgatcagcctcgactgtgccttctagttgccagccatctgttgtttgcccctcccccgtgccttccttgaccctggaaggtgccactcccactgtcctttcctaataaaatgaggaaattgcatcgcattgtctgagtaggtgtcattctattctggggggtgggggtggggcaggacagcaagggggaggattgggaagacaatagcaggcatgctggggatgcggtgggctctatggcttctgaggcggaaagaaccagctggggctctagggggtatccccacgcgccctgtagcggcgcattaagcgcggcgggtgtggtggttacgcgcagcgtgaccgctacacttgccagcgccctagcgcccgctcctttcgctttcttcccttcctttctcgccacgttcgccggctttccccgtcaagctctaaatcgggggctccctttagggttccgatttagtgctttacggcacctcgaccccaaaaaacttgattagggtgatggttcacgtagtgggccatcgccctgatagacggtttttcgccctttgacgttggagtccacgttctttaatagtggactcttgttccaaactggaacaacactcaaccctatctcggtctattcttttgatttataagggattttgccgatttcggcctattggttaaaaaatgagctgatttaacaaaaatttaacgcgaattaattctgtggaatgtgtgtcagttagggtgtggaaagtccccaggctccccagcaggcagaagtatgcaaagcatgcatctcaattagtcagcaaccaggtgtggaaagtccccaggctccccagcaggcagaagtatgcaaagcatgcatctcaattagtcagcaaccatagtcccgcccctaactccgcccatcccgcccctaactccgcccagttccgcccattctccgccccatggctgactaattttttttatttatgcagaggccgaggccgcctctgcctctgagctattccagaagtagtgaggaggcttttttggaggcctaggcttttgcaaaaagctcccgggagcttgtatatccattttcggatctgatcagcacagcttaccatgaccgagtacaagcccacggtgcgcctcgccacccgcgacgacgtccccagggccgtacgcaccctcgccgccgcgttcgccgactaccccgccacgcgccacaccgtcgatccggaccgccacatcgagcgggtcaccgagctgcaagaactcttcctcacgcgcgtcgggctcgacatcggcaaggtgtgggtcgcggacgacggcgccgccgtggcggtctggaccacgccggagagcgtcgaagcgggggcggtgttcgccgagatcggcccgcgcatggccgagttgagcggttcccggctggccgcgcagcaacagatggaaggcctcctggcgccgcaccggcccaaggagcccgcgtggttcctggccaccgtcggcgtctcgcccgaccaccagggcaagggtctgggcagcgccgtcgtgctccccggagtggaggcggccgagcgcgccggggtgcccgccttcctggagacctccgcgccccgcaacctccccttctacgagcggctcggcttcaccgtcaccgccgacgtcgaggtgcccgaaggaccgcgcacctggtgcatgacccgcaagcccggtgcctgacgcccgccccacgacccgcagcgcccgaccgaaaggagcgcacgaccccatgcatcggtgctacgagatttcgattccaccgccgccttctatgaaaggttgggcttcggaatcgttttccgggacgccggctggatgatcctccagcgcggggatctcatgctggagttcttcgcccaccccaacttgtttattgcagcttataatggttacaaataaagcaatagcatcacaaatttcacaaataaagcatttttttcactgcattctagttgtggtttgtccaaactcatcaatgtatcttatcatgtctgtataccgtcgacctctagctagagcccgcggatcgatggatccattcatgaatgaattcatgtcgacatactagtgcgcgcgttgacattgattattgactagttattaatagtaatcaattacggggtcattagttcatagcccatatatggagttccgcgttacataacttacggtaaatggcccgcctggctgaccgcccaacgacccccgcccattgacgtcaataatgacgtatgttcccatagtaacgccaatagggactttccattgacgtcaatgggtggactatttacggtaaactgcccacttggcagtacatcaagtgtatcatatgccaagtacgccccctattgacgtcaatgacggtaaatggcccgcctggcattatgcccagtacatgaccttatgggactttcctacttggcagtacatctacgtattagtcatcgctattaccatggtgatgcggttttggcagtacatcaatgggcgtggatagcggtttgactcacggggatttccaagtctccaccccattgacgtcaatgggagtttgttttggcaccaaaatcaacgggactttccaaaatgtcgtaacaactccgccccattgacgcaaatgggcggtaggcgtgtacggtgggaggtctatataagcagagctctctggctaactagagaacccactgcttactggcttatcgaaattaatacgactcactatagggagacccaagcttggtaccgagctcggatccactagtaacggccgccagtgtgctggaattcggcttggggatatccaccatggagacagacacactcctgctatgggtactgctgctctgggttccaggttccactggtgatgttaacgaacccaagacaccaaaaccacaaccacaaccacaaccacaacccaatcctacaacagaatccaagtgtcccaaatgtccagcccctgagctcctgggagggccctcagtcttcatcttccccccgaaacccaaggacgtcctctccatttctgggaggcccgaggtcacgtgcgttgtggtagacgtgggccaggaagaccccgaggtcagtttcaactggtacattgatggcgctgaggtgcgaacggccaacacgaggccaaaagaggaacagttcaacagcacgtaccgcgtggtcagcgtcctgcccatccagcaccaggactggctgacggggaaggaattcaagtgcaaggtcaacaacaaagctctcccggcccccatcgagaagaccatctccaaggccaaagggcagacccgggagccgcaggtgtacgccctggccccacaccgggaagagctggccaaggacaccgtgagcgtaacatgcctggtcaaaggcttctacccacctgatatcaacgttgagtggcagaggaaccggcagccggagccagagggcacctacgccaccacgccgccacagctggacaacgacgggacctacttcctctacagcaagctctcggtgggaaagaacacgtggcagcggggagaaaccttcacctgtgtggtgatgcacgagaccctgcacaaccactacacccagaaatccatctcccagtcttaaaacacggaaggagacaataccggaaggaacccgcgctatgacggcaataaaaagacagaataaaacgcacgggtgttgggtcgtttgttcataaacgcggggttcggtccccatcaactagaatgctaactagttaaaagttttgttactttatagaagaaattttgagtttttgtttttttttaataaataaataaacataaataaattgtttgttgaatttattattagtatgtaagtgtaaatataataaaacttaatatctattcaaattaataaataaacctcgatatacagaccgataaaacacatgcgtcaattttacgcatgattatctttaacgtacgtcacaatatgattatctttctagggttaatctagtatacgcgtatgcggccgcttaattaatccagcttttgttccctttagtgagggttaattgcgcgcttggcgtaatcatggtcatagctgtttcctgtgtgaaattgttatccgctcacaattccacacaacatacgagccggaagcataaagtgtaaagcctggggtgcctaatgagtgagctaactcacattaattgcgttgcgctcactgcccgctttccagtcgggaaacctgtcgtgccagctgcattaatgaatcggccaacgcgcggggagaggcggtttgcgtattgggcgctcttccgcttcctcgctcactgactcgctgcgctcggtcgttcggctgcggcgagcggtatcagctcactcaaaggcggtaatacggttatccacagaatcaggggataacgcaggaaagaacatgtgagcaaaaggccagcaaaaggccaggaaccgtaaaaaggccgcgttgctggcgtttttccataggctccgcccccctgacgagcatcacaaaaatcgacgctcaagtcagaggtggcgaaacccgacaggactataaagataccaggcgtttccccctggaagctccctcgtgcgctctcctgttccgaccctgccgcttaccggatacctgtccgcctttctcccttcgggaagcgtggcgctttctcatagctcacgctgtaggtatctcagttcggtgtaggtcgttcgctccaagctgggctgtgtgcacgaaccccccgttcagcccgaccgctgcgccttatccggtaactatcgtcttgagtccaacccggtaagacacgacttatcgccactggcagcagccactggtaacaggattagcagagcgaggtatgtaggcggtgctacagagttcttgaagtggtggcctaactacggctacactagaaggacagtatttggtatctgcgctctgctgaagccagttaccttcggaaaaagagttggtagctcttgatccggcaaacaaaccaccgctggtagcggtggtttttttgtttgcaagcagcagattacgcgcagaaaaaaaggatctcaagaagatcctttgatcttttctacggggtctgacgctcagtggaacgaaaactcacgttaagggattttggtcatgagattatcaaaaaggatcttcacctagatccttttaaattaaaaatgaagttttaaatcaatctaaagtatatatgagtaaacttggtctgacagttaccaatgcttaatcagtgaggcacctatctcagcgatctgtctatttcgttcatccatagttgcctgactccccgtcgtgtagataactacgatacgggagggcttaccatctggccccagtgctgcaatgataccgcgagacccacgctcaccggctccagatttatcagcaataaaccagccagccggaagggccgagcgcagaagtggtcctgcaactttatccgcctccatccagtctattaattgttgccgggaagctagagtaagtagttcgccagttaatagtttgcgcaacgttgttgccattgctacaggcatcgtggtgtcacgctcgtcgtttggtatggcttcattcagctccggttcccaacgatcaaggcgagttacatgatcccccatgttgtgcaaaaaagcggttagctccttcggtcctccgatcgttgtcagaagtaagttggccgcagtgttatcactcatggttatggcagcactgcataattctcttactgtcatgccatccgtaagatgcttttctgtgactggtgagtactcaaccaagtcattctgagaatagtgtatgcggcgaccgagttgctcttgcccggcgtcaatacgggataataccgcgccacatagcagaactttaaaagtgctcatcattggaaaacgttcttcggggcgaaaactctcaaggatcttaccgctgttgagatccagttcgatgtaacccactcgtgcacccaactgatcttcagcatcttttactttcaccagcgtttctgggtgagcaaaaacaggaaggcaaaatgccgcaaaaaagggaataagggcgacacggaaatgttgaatactcatactcttcctttttcaatattattgaagcatttatcagggttattgtctcatgagcggatacatatttgaatgtatttagaaaaataaacaaataggggttccgcgcacatttccccgaaaagtgccac

SEQ ID NO: 16 - protein, 19 aa, Mouse
MGWSCIILFLVATATGVHS

SEQ ID NO: 17 - protein, 21 aa, Mouse
METDTLLLWVLLLWVPGSTGD

SEQ ID NO: 18 - protein, 24 aa, Human
MALWMRLLPLLALLALWGPDPAAA

SEQ ID NO: 19 - protein, 20 aa, Human
MYRMQLLSCIALSLALVTNS

SEQ ID NO: 20 - protein, 15 aa, Human
MNLLLILTFVAAAVA